European Patent Specification EP 3 702 462 B1, published October 9, 2024. Title: FC-BINDING PROTEIN WITH IMPROVED ALKALINE STABILITY, METHOD FOR PRODUCING SAID PROTEIN, ANTIBODY ADSORBENT USING SAID PROTEIN, AND METHOD FOR SEPARATING ANTIBODY USING SAID ADSORBENT. Applicant: TOSOH Corporation. The sequence listing filed with the application follows.

SEQUENCE LISTING (29 sequences)

SEQ ID NO: 1 - protein, 254 aa, Homo sapiens
  ref <308>: UniProt P08637
  ref <309>: 1990-08-01
  ref <313>: (1)..(254)
MWQLLLPTALLLLVSAGMRTEDLPKAVVFLEPQWYRVLEKDSVTLKCQGAYSPEDNSTQWFHNESLISSQASSYFIDAATVDDSGEYRCQTNLSTLSDPVQLEVHIGWLLLQAPRWVFKEEDPIHLRCHSWKNTALHKVTYLQNGKGRKYFHHNSDFYIPKATLKDSGSYFCRGLFGSKNVSSETVNITITQGLAVSTISSFFPPGYQVSFCLVMVLLFAVDTGLYFSVKTNIRSSTRDWKDHKFKWRKDPQDK

SEQ ID NO: 2 - DNA, 20 bp, Artificial Sequence
  Oligonucleotide
taatacgactcactataggg

SEQ ID NO: 3 - DNA, 19 bp, Artificial Sequence
  Oligonucleotide
tatgctagttattgctcag

SEQ ID NO: 4 - protein, 216 aa, Artificial Sequence
  MalE-CD16a-6His
MKIKTGARILALSALTTMMFSASALAKIEEAMGMRTEDLPKAVVFLEPQWYRVLEKDSVTLKCQGAYSPEDNSTQWFHNESLISSQASSYFIDAATVDDSGEYRCQTNLSTLSDPVQLEVHIGWLLLQAPRWVFKEEDPIHLRCHSWKNTALHKVTYLQNGKGRKYFHHNSDFYIPKATLKDSGSYFCRGLVGSKNVSSETVNITITQGGHHHHHH

SEQ ID NO: 5 - protein, 216 aa, Artificial Sequence
  FcR35c
MKIKTGARILALSALTTMMFSASALAKIEEAMGMRTGDMPKAEVILEPPWNRVLEQDSVTLKCRGAHSPDDDSTQWFHNESLIPSQASSFIIDSASVEDSGEYRCQTSLSTLSEPVLLEVHIGWLLLQAPRWEFVEGEPIHLRCHSWRNTALHKVMFLQNGKVRKYFHHNSDFVIPKATLEDSGSYSCRGLVGRKNVSSEAVEITVTPGGHHHHHH

SEQ ID NO: 6 - DNA, 648 bp, Artificial Sequence
  Polynucleotide encoding FcR35c
atgaaaataaaaacaggtgcacgcatcctcgcattatccgcattaacgacgatgatgttttccgcctcggctctcgccaaaatcgaagaagccatgggcatgcgtaccggagatatgccgaaagcggaggtgattctggaaccgccgtggaatcgcgtgctggagcaagattcagtgacccttaaatgccggggcgcgcatagcccggatgatgacagcacccagtggttccacaatgaaagcctgattcccagccaggcgagcagcttcattattgattcggcgtcggtggaagatagcggcgaatatcgttgccagaccagcctgagcaccctgagcgaaccggtgctgctggaggtgcacatcgggtggcttctgttacaggctccacggtgggagttcgtagagggggaaccgattcatctgcggtgtcactcctggaggaataccgccctgcataaagtgatgttcctgcaaaacggcaaggtccgcaagtatttccaccacaactccgacttcgttattcccaaagcgacgctggaggacagcggcagctattcctgccgtgggctggtgggcagaaaaaatgtgagcagcgaggccgtggaaattaccgttaccccagggggccatcatcatcatcatcat

SEQ ID NO: 7 - protein, 216 aa, Artificial Sequence
  FcR35d
MKIKTGARILALSALTTMMFSASALAKIEEAMGMRTGDMPKAEVILEPPWNRVLEQDSVTLKCRGAHSPDDDSTQWFHNERLIPSQASSFIIDSASVDDSGEYRCQTSLSTLSDPVQLEVHIGWLLLQAPRWEFVEGEPIHLRCHSWRNTALHKVMFLQNGKVRKYFHHNSDFVIPKATLEDSGSYSCRGLVGRKKVSSGAVDITVTQGGHHHHHH

SEQ ID NO: 8 - DNA, 648 bp, Artificial Sequence
  Polynucleotide encoding FcR35d
atgaaaataaaaacaggtgcacgcatcctcgcattatccgcattaacgacgatgatgttttccgcctcggctctcgccaaaatcgaagaagccatgggcatgcgtaccggagatatgccgaaagcggaggtgattctggaaccgccgtggaatcgcgtgctggagcaagattcagtgacccttaaatgccggggcgcgcatagcccggatgatgacagcacccagtggttccacaatgaacgcctgattcccagccaggcgagcagcttcattattgattcggcgtcggtggatgatagcggcgaatatcgttgccagaccagcctgagcaccctgagcgatccggtgcagctggaggtgcacatcgggtggcttctgttacaggctccacggtgggagttcgtagagggggaaccgattcatctgcggtgtcactcctggaggaataccgccctgcataaagtgatgttcctgcaaaacggcaaggtccgcaagtatttccaccacaactccgacttcgttattcccaaagcgacgctggaggacagcggcagctattcctgccgtgggctggtgggcagaaaaaaggtgagcagcggggccgtggacattaccgttacccaagggggccatcatcatcatcatcat

SEQ ID NO: 9 - protein, 216 aa, Artificial Sequence
  FcR36i
MKIKTGARILALSALTTMMFSASALAKIEEAMGMRTGDMPKAEVILEPPWNRVLEQDSVTLKCRGAHSPDDDSTQWFHNERLIPSQASSFIIDSASVDDSGEYRCQTSLSTLSDPVQLEVHIGWLLLQAPRWEFVEGEPIHLRCHSWRNTALHKVMFLQNGKVRKYFHHNSDFVIPKATLEDSGSYSCRGLIGRKKVSSGAVDITVTQGGHHHHHH

SEQ ID NO: 10 - DNA, 648 bp, Artificial Sequence
  Polynucleotide encoding FcR36i
atgaaaataaaaacaggtgcacgcatcctcgcattatccgcattaacgacgatgatgttttccgcctcggctctcgccaaaatcgaagaagccatgggcatgcgtaccggagatatgccgaaagcggaggtgattctggaaccgccgtggaatcgcgtgctggagcaagattcagtgacccttaaatgccggggcgcgcatagcccggatgatgacagcacccagtggttccacaatgaacgcctgattcccagccaggcgagcagcttcattattgattcggcgtcggtggatgatagcggcgaatatcgttgccagaccagcctgagcaccctgagcgatccggtgcagctggaggtgcacatcgggtggcttctgttacaggctccacggtgggagttcgtagagggggaaccgattcatctgcggtgtcactcctggaggaataccgccctgcataaagtgatgttcctgcaaaacggcaaggtccgcaagtatttccaccacaactccgacttcgttattcccaaagcgacgctggaggacagcggcagctattcctgccgtgggctgattggcagaaaaaaggtgagcagcggggccgtggacattaccgttacccaagggggccatcatcatcatcatcat

SEQ ID NO: 11 - protein, 216 aa, Artificial Sequence
  FcR36a
MKIKTGARILALSALTTMMFSASALAKIEEAMGMRTGDMPKAEVILEPPWNRVLEQDSVTLKCRGAHSPDDDSTQWFHNERLIPSQASSFIIDSASVDDSGEYRCQTSLSTLSDPVQLEVHIGWLLLQAPRWEFVEGEPIHLRCHSWRNTALHKVMFLQNGKVRKYFHHNSDFVIPKATLEDSGSYSCRGLAGRKKVSSGAVDITVTQGGHHHHHH

SEQ ID NO: 12 - DNA, 648 bp, Artificial Sequence
  Polynucleotide encoding FcR36a
atgaaaataaaaacaggtgcacgcatcctcgcattatccgcattaacgacgatgatgttttccgcctcggctctcgccaaaatcgaagaagccatgggcatgcgtaccggagatatgccgaaagcggaggtgattctggaaccgccgtggaatcgcgtgctggagcaagattcagtgacccttaaatgccggggcgcgcatagcccggatgatgacagcacccagtggttccacaatgaacgcctgattcccagccaggcgagcagcttcattattgattcggcgtcggtggatgatagcggcgaatatcgttgccagaccagcctgagcaccctgagcgatccggtgcagctggaggtgcacatcgggtggcttctgttacaggctccacggtgggagttcgtagagggggaaccgattcatctgcggtgtcactcctggaggaataccgccctgcataaagtgatgttcctgcaaaacggcaaggtccgcaagtatttccaccacaactccgacttcgttattcccaaagcgacgctggaggacagcggcagctattcctgccgtgggctggcgggcagaaaaaaggtgagcagcggggccgtggacattaccgttacccaagggggccatcatcatcatcatcat

SEQ ID NO: 13 - DNA, 53 bp, Artificial Sequence
  Oligonucleotide
catatgaaaataaaaacaggtgcacgcatcctcgcattatccgcattaacgac

SEQ ID NO: 14 - DNA, 65 bp, Artificial Sequence
  Oligonucleotide
cccaagcttatccgcaggtatcgttgcggcacccttgggtaacggtaatgtccacggccccgctg

SEQ ID NO: 15 - DNA, 19 bp, Artificial sequence
  Oligonucleotide
tgtggtatggctgtgcagg

SEQ ID NO: 16 - DNA, 18 bp, Artificial sequence
  Oligonucleotide
tcggcatggggtcaggtg

SEQ ID NO: 17 - protein, 207 aa, Artificial sequence
  FcR36i_Cys
MKYLLSTAAAGLLLLAAQPAMAMGMRTGDMPKAEVILEPPWNRVLEQDSVTLKCRGAHSPDDDSTQWFHNERLIPSQASSFIIDSASVDDSGEYRCQTSLSTLSDPVQLEVHIGWLLLQAPRWEFVEGEPIHLRCHSWRNTALHKVMFLQNGKVRKYFHHNSDFVIPKATLEDSGSYSCRGLIGRKKVSSGAVDITVTQGCRNDTCG

SEQ ID NO: 18 - DNA, 621 bp, Artificial sequence
  Polynucleotide encoding FcR36i_Cys
atgaaatacctgctgtcgaccgctgctgctggtctgctgctcctcgctgcccagccggcgatggccatgggcatgcgtaccggagatatgccgaaagcggaggtgattctggaaccgccgtggaatcgcgtgctggagcaagattcagtgacccttaaatgccggggcgcgcatagcccggatgatgacagcacccagtggttccacaatgaacgcctgattcccagccaggcgagcagcttcattattgattcggcgtcggtggatgatagcggcgaatatcgttgccagaccagcctgagcaccctgagcgatccggtgcagctggaggtgcacatcgggtggcttctgttacaggctccacggtgggagttcgtagagggggaaccgattcatctgcggtgtcactcctggaggaataccgccctgcataaagtgatgttcctgcaaaacggcaaggtccgcaagtatttccaccacaactccgacttcgttattcccaaagcgacgctggaggacagcggcagctattcctgccgtgggctgattggcagaaaaaaggtgagcagcggggccgtggacattaccgttacccaagggtgccgcaacgatacctgcgga

SEQ ID NO: 19 - protein, 254 aa, Homo sapiens
  ref <308>: GenBank AAH17865.1
MWQLLLPTALLLLVSAGMRTEDLPKAVVFLEPQWYRVLEKDSVTLKCQGAYSPEDNSTQWFHNESLISSQASSYFIDAATVDDSGEYRCQTNLSTLSDPVQLEVHIGWLLLQAPRWVFKEEDPIHLRCHSWKNTALHKVTYLQNGKGRKYFHHNSDFYIPKATLKDSGSYFCRGLVGSKNVSSETVNITITQGLAVSTISSFFPPGYQVSFCLVMVLLFAVDTGLYFSVKTNIRSSTRDWKDHKFKWRKDPQDK

SEQ ID NO: 20 - protein, 216 aa, Artificial Sequence
  FcR9
MKIKTGARILALSALTTMMFSASALAKIEEAMGMRTEDLPKAEVILEPQWNRVLEKDSVTLKCRGAYSPEDNSTQWFHNESLISSQASSYLIDAATVDDSGEYRCQTSLSTLSDPVQLEVHIGWLLLQAPRWEFKEGDPIHLRCHSWKNTALHKVTYLQNGKGRKYFHHNSDFYIPKATLKDSGSYSCRGLVGSKNVSSETVNITITQGGHHHHHH

SEQ ID NO: 21 - DNA, 648 bp, Artificial Sequence
  Polynucleotide encoding FcR9
atgaaaataaaaacaggtgcacgcatcctcgcattatccgcattaacgacgatgatgttttccgcctcggctctcgccaaaatcgaagaagccatgggcatgcgtaccgaagatctgccgaaagcggaggtgattctggaaccgcagtggaatcgcgtgctggagaaagattctgtgacccttaaatgccggggcgcgtatagcccggaagataacagcacccagtggttccacaatgaaagcctgatttccagccaggcgagcagctaccttattgatgcggcgacggtggatgatagcggcgaatatcgttgccagaccagcctgagcaccctgagcgatccggtgcagctggaggtgcacatcgggtggcttctgttacaggctccacggtgggagttcaaagagggggatccgattcatctgcggtgtcactcctggaagaataccgccctgcataaagtgacctacctgcaaaacggcaagggccgcaagtatttccaccacaactccgacttctatattcccaaagcgacgctgaaggacagcggcagctattcctgccgtgggctggtgggcagcaaaaatgtgagcagcgagaccgtgaatattaccattacccaagggggccatcatcatcatcatcat

SEQ ID NO: 22 - DNA, 30 bp, Artificial Sequence
  Oligonucleotide
  misc_feature (15)..(16): n is a, c, g, or t
catttttgctgccmnncagcccacggcagg

SEQ ID NO: 23 - DNA, 30 bp, Artificial Sequence
  Artificial sequence
  misc_feature (15)..(16): n is a, c, g, or t
cctgccgtgggctgnnkggcagcaaaaatg

SEQ ID NO: 24 - protein, 216 aa, Artificial Sequence
  FcR9_I
MKIKTGARILALSALTTMMFSASALAKIEEAMGMRTEDLPKAEVILEPQWNRVLEKDSVTLKCRGAYSPEDNSTQWFHNESLISSQASSYLIDAATVDDSGEYRCQTSLSTLSDPVQLEVHIGWLLLQAPRWEFKEGDPIHLRCHSWKNTALHKVTYLQNGKGRKYFHHNSDFYIPKATLKDSGSYSCRGLIGSKNVSSETVNITITQGGHHHHHH

SEQ ID NO: 25 - DNA, 648 bp, Artificial Sequence
  Polynucleotide encoding FcR9_I
atgaaaataaaaacaggtgcacgcatcctcgcattatccgcattaacgacgatgatgttttccgcctcggctctcgccaaaatcgaagaagccatgggcatgcgtaccgaagatctgccgaaagcggaggtgattctggaaccgcagtggaatcgcgtgctggagaaagattctgtgacccttaaatgccggggcgcgtatagcccggaagataacagcacccagtggttccacaatgaaagcctgatttccagccaggcgagcagctaccttattgatgcggcgacggtggatgatagcggcgaatatcgttgccagaccagcctgagcaccctgagcgatccggtgcagctggaggtgcacatcgggtggcttctgttacaggctccacggtgggagttcaaagagggggatccgattcatctgcggtgtcactcctggaagaataccgccctgcataaagtgacctacctgcaaaacggcaagggccgcaagtatttccaccacaactccgacttctatattcccaaagcgacgctgaaggacagcggcagctattcctgccgtgggctgattggcagcaaaaatgtgagcagcgagaccgtgaatattaccattacccaagggggccatcatcatcatcatcat

SEQ ID NO: 26 - protein, 216 aa, Artificial Sequence
  FcR9_A
MKIKTGARILALSALTTMMFSASALAKIEEAMGMRTEDLPKAEVILEPQWNRVLEKDSVTLKCRGAYSPEDNSTQWFHNESLISSQASSYLIDAATVDDSGEYRCQTSLSTLSDPVQLEVHIGWLLLQAPRWEFKEGDPIHLRCHSWKNTALHKVTYLQNGKGRKYFHHNSDFYIPKATLKDSGSYSCRGLAGSKNVSSETVNITITQGGHHHHHH

SEQ ID NO: 27 - DNA, 648 bp, Artificial Sequence
  Polynucleotide encoding FcR9_A
atgaaaataaaaacaggtgcacgcatcctcgcattatccgcattaacgacgatgatgttttccgcctcggctctcgccaaaatcgaagaagccatgggcatgcgtaccgaagatctgccgaaagcggaggtgattctggaaccgcagtggaatcgcgtgctggagaaagattctgtgacccttaaatgccggggcgcgtatagcccggaagataacagcacccagtggttccacaatgaaagcctgatttccagccaggcgagcagctaccttattgatgcggcgacggtggatgatagcggcgaatatcgttgccagaccagcctgagcaccctgagcgatccggtgcagctggaggtgcacatcgggtggcttctgttacaggctccacggtgggagttcaaagagggggatccgattcatctgcggtgtcactcctggaagaataccgccctgcataaagtgacctacctgcaaaacggcaagggccgcaagtatttccaccacaactccgacttctatattcccaaagcgacgctgaaggacagcggcagctattcctgccgtgggctggcgggcagcaaaaatgtgagcagcgagaccgtgaatattaccattacccaagggggccatcatcatcatcatcat

SEQ ID NO: 28 - protein, 216 aa, Artificial Sequence
  FcR9_Y
MKIKTGARILALSALTTMMFSASALAKIEEAMGMRTEDLPKAEVILEPQWNRVLEKDSVTLKCRGAYSPEDNSTQWFHNESLISSQASSYLIDAATVDDSGEYRCQTSLSTLSDPVQLEVHIGWLLLQAPRWEFKEGDPIHLRCHSWKNTALHKVTYLQNGKGRKYFHHNSDFYIPKATLKDSGSYSCRGLYGSKNVSSETVNITITQGGHHHHHH

SEQ ID NO: 29 - DNA, 648 bp, Artificial Sequence
  Polynucleotide encoding FcR9_Y
atgaaaataaaaacaggtgcacgcatcctcgcattatccgcattaacgacgatgatgttttccgcctcggctctcgccaaaatcgaagaagccatgggcatgcgtaccgaagatctgccgaaagcggaggtgattctggaaccgcagtggaatcgcgtgctggagaaagattctgtgacccttaaatgccggggcgcgtatagcccggaagataacagcacccagtggttccacaatgaaagcctgatttccagccaggcgagcagctaccttattgatgcggcgacggtggatgatagcggcgaatatcgttgccagaccagcctgagcaccctgagcgatccggtgcagctggaggtgcacatcgggtggcttctgttacaggctccacggtgggagttcaaagagggggatccgattcatctgcggtgtcactcctggaagaataccgccctgcataaagtgacctacctgcaaaacggcaagggccgcaagtatttccaccacaactccgacttctatattcccaaagcgacgctgaaggacagcggcagctattcctgccgtgggctgtatggcagcaaaaatgtgagcagcgagaccgtgaatattaccattacccaagggggccatcatcatcatcatcat